European Patent Application EP 4 732 909 A2, published April 29, 2026. Title: ANTI-CD154 ANTIBODY HAVING IMPROVED BINDING, FUNCTIONAL AND SAFETY CHARACTERISTICS AND USE IN HUMAN IMMUNOTHERAPY. Applicant: Immunext, Inc. Application EP. The sequence listing filed with the application follows.

SEQUENCE LISTING (34 sequences)

SEQ ID NO: 1 - protein, 120 aa, synthetic construct
  REGION 1..120: note = INX021 Variable Heavy
EVQLQESGPGLVKPSETLSLTCTVSGDSITNGFWIWIRKPPGNKLEYMGYISYSGSTYYNPSLKSRISISRDTSKNQFSLKLSSVTAADTGVYYCAYRSYGRTPYYFDYWGQGTTLTVSS

SEQ ID NO: 2 - protein, 107 aa, synthetic construct
  REGION 1..107: note = INX021 Variable Light
DIVMTQSPSFLSASVGDRVTITCKASSNLGHAVAWYQQKPGKSPKLLIYSASNRYTGVPDRFSGSGSGTDFTLTISSLQPEDFADYFCQQYDDYPYTFGGGTKLEIK

SEQ ID NO: 3 - protein, 330 aa, synthetic construct
  REGION 1..330: note = INX021 Constant Heavy
ASTKGPSVFPLAPSSKSTSGGTAALGCLVKDYFPEPVTVSWNSGALTSGVHTFPAVLQSSGLYSLSSVVTVPSSSLGTQTYICNVNHKPSNTKVDKKAEPKSCDKTHTCPPCPAPELLGGPSVFLFPPKPKDTLMISRTPEVTCVVVDVSHRDPEVKFNWYVDGVEVHNAKTKPREEQYNSTYRVVSVLTVLHQDWLNGKEYKCAVSNKALPAPIEKTISKAKGQPREPQVYTLPPSRDELTKNQVSLTCLVKGFYPSDIAVEWESNGQPENNYKTTPPVLDSDGSFFLYSKLTVDKSRWQQGNVFSCSVMHEALHNHYTQKSLSLSPGK

SEQ ID NO: 4 - protein, 107 aa, synthetic construct [sequence omitted]

SEQ ID NO: 5 - protein, 10 aa, Mus musculus
GDSITNGFWI

SEQ ID NO: 6 - protein, 9 aa, Mus musculus
YISYSGSTY

SEQ ID NO: 7 - protein, 13 aa, Mus musculus
YRSYGRTPYYFDY

SEQ ID NO: 8 - protein, 11 aa, Mus musculus
KASSNLGHAVA

SEQ ID NO: 9 - protein, 7 aa, Mus musculus
SASNRYT

SEQ ID NO: 10 - protein, 9 aa, Mus musculus
QQYDDYPYT

SEQ ID NO: 11 - protein, 330 aa, Homo sapiens [sequence omitted]

SEQ ID NO: 12 - protein, 330 aa, synthetic construct [sequence omitted]

SEQ ID NO: 13 - protein, 330 aa, Mus musculus; identical to SEQ ID NO: 3

SEQ ID NO: 14 - protein, 330 aa, synthetic construct [sequence omitted]

SEQ ID NO: 15 - protein, 120 aa, synthetic construct
  REGION 1..120: note = IDEC-131 Variable Heavy-Chain Sequence
EVQLQESGPGLVKPSETLSLTCTVSGDSITNGFWIWIRKPPGNKLEYMGYISYSGSTYYNPSLKSRISISRDTSKNQFSLKLSSVTAADTGVYYCACRSYGRTPYYFDFWGQGTTLTVSS

SEQ ID NO: 16 - protein, 120 aa, Mus musculus
EVQLQESGPGLVKPSETLSLTCTVSGDSITNGFWIWIRKPPGNKLEYMGYISYSGSTYYNPSLKSRISISRDTSKNQFSLKLSSVTAADTGVYYCAYRSYGRTPYYFDFWGQGTTLTVSS

SEQ ID NO: 17 - protein, 120 aa, Homo sapiens; identical to SEQ ID NO: 1

SEQ ID NO: 18 - protein, 120 aa, synthetic construct; identical to SEQ ID NO: 16
  REGION 1..120: note = Variable heavy-chain sequence consensus

SEQ ID NO: 19 - protein, 107 aa, Mus musculus
DIVMTQSPSFLSASVGDRVTITCKASQNVITAVAWYQQKPGKSPKLLIYSASNRYTGVPDRFSGSGSGTDFTLTISSLQPEDFADYFCQQYDDYPYTFGGGTKLEIK

SEQ ID NO: 20 - protein, 107 aa, synthetic construct
  REGION 1..107: note = IDEC_AB2-IMX variable light chain sequence
DIVMTQSPSFLSASVGDRVTITCKASQNVITAVAWYQQKPGKSPKLLIYSASNRYTGVPDRFSGSGSGTDFTLTISSLQPEDFADYFCQQYNSYPYTFGGGTKLEIK

SEQ ID NO: 21 - protein, 107 aa, synthetic construct
  REGION 1..107: note = Variable light-chain sequence 30
DIVMTQSPSFLSASVGDRVTITCKAGHSLGTAVAWYQQKPGKSPKLLIYSASNRYTGVPDRFSGSGSGTDFTLTISSLQPEDFADYFCQQYDDYPYTFGGGTKLEIK

SEQ ID NO: 22 - protein, 107 aa, synthetic construct
  REGION 1..107: note = Variable light-chain sequence 25
DIVMTQSPSFLSASVGDRVTITCKASQNLNHAVAWYQQKPGKSPKLLIYSASNRYTGVPDRFSGSGSGTDFTLTISSLQPEDFADYFCQQYDDYPYTFGGGTKLEIK

SEQ ID NO: 23 - protein, 107 aa, synthetic construct
  REGION 1..107: note = Variable light-chain sequence 22
DIVMTQSPSFLSASVGDRVTITCKASSNLGNAVAWYQQKPGKSPKLLIYSASNRYTGVPDRFSGSGSGTDFTLTISSLQPEDFADYFCQQYDDYPYTFGGGTKLEIK

SEQ ID NO: 24 - protein, 107 aa, synthetic construct; identical to SEQ ID NO: 2
  REGION 1..107: note = Variable light-chain sequence 21

SEQ ID NO: 25 - protein, 107 aa, synthetic construct
  REGION 1..107: note = Variable light-chain sequence 28
DIVMTQSPSFLSASVGDRVTITCKAPSSLGHAVAWYQQKPGKSPKLLIYSASNRYTGVPDRFSGSGSGTDFTLTISSLQPEDFADYFCQQYDDYPYTFGGGTKLEIK

SEQ ID NO: 26 - protein, 107 aa, synthetic construct
  REGION 1..107: note = Variable light-chain sequence 23
DIVMTQSPSFLSASVGDRVTITCKGSSPLGHAVAWYQQKPGKSPKLLIYSASNRYTGVPDRFSGSGSGTDFTLTISSLQPEDFADYFCQQYDDYPYTFGGGTKLEIK

SEQ ID NO: 27 - protein, 107 aa, synthetic construct
  REGION 1..107: note = Variable light-chain sequence 31
DIVMTQSPSFLSASVGDRVTITCKANQPLGHAVAWYQQKPGKSPKLLIYSASNRYTGVPDRFSGSGSGTDFTLTISSLQPEDFADYFCQQYDDYPYTFGGGTKLEIK

SEQ ID NO: 28 - protein, 107 aa, synthetic construct
  REGION 1..107: note = Variable light-chain sequence 29
DIVMTQSPSFLSASVGDRVTITCKGNQPLGHAVAWYQQKPGKSPKLLIYSASNRYTGVPDRFSGSGSGTDFTLTISSLQPEDFADYFCQQYDDYPYTFGGGTKLEIK

SEQ ID NO: 29 - protein, 107 aa, synthetic construct
  REGION 1..107: note = Variable light-chain sequence 27
DIVMTQSPSFLSASVGDRVTITCKASQHLGHAVAWYQQKPGKSPKLLIYSASNRYTGVPDRFSGSGSGTDFTLTISSLQPEDFADYFCQQYDDYPYTFGGGTKLEIK

SEQ ID NO: 30 - protein, 107 aa, synthetic construct
  REGION 1..107: note = Variable light-chain sequence 26
DIVMTQSPSFLSASVGDRVTITCKASQHLGTAVAWYQQKPGKSPKLLIYSASNRYTGVPDRFSGSGSGTDFTLTISSLQPEDFADYFCQQYDDYPYTFGGGTKLEIK

SEQ ID NO: 31 - protein, 107 aa, synthetic construct
  REGION 1..107: note = Variable light-chain sequence 24
DIVMTQSPSFLSASVGDRVTITCKAPQNLGTAVAWYQQKPGKSPKLLIYSASNRYTGVPDRFSGSGSGTDFTLTISSLQPEDFADYFCQQYDDYPYTFGGGTKLEIK

SEQ ID NO: 32 - protein, 107 aa, synthetic construct
  REGION 1..107: note = Variable light-chain sequence consensus
DIVMTQSPSFLSASVGDRVTITCKASQNLGHAVAWYQQKPGKSPKLLIYSASNRYTGVPDRFSGSGSGTDFTLTISSLQPEDFADYFCQQYDDYPYTFGGGTKLEIK

SEQ ID NO: 33 - protein, 450 aa, synthetic construct
  REGION 1..450: note = INX021 Variable Heavy with CDRs, affinity maturation mutated residues and Fc mutations
EVQLQESGPGLVKPSETLSLTCTVSGDSITNGFWIWIRKPPGNKLEYMGYISYSGSTYYNPSLKSRISISRDTSKNQFSLKLSSVTAADTGVYYCAYRSYGRTPYYFDINGQGTTLTVSSASTKGPSVFPLAPSSKSTSGGTAALGCLVKDYFPEPVTVSWNSGALTSGVHTFPAVLQSSGLYSLSSVVTVPSSSLGTQTYICNVNHKPSNTKVDKKAEPKSCDKTHTCPPCPAPELLGGPSVFLFPPKPKDTLMISRTPEVTCVVVDVSHRDPEVKFNWYVDGVEVHNAKTKPREEQYNSTYRVVSVLTVLHQDWLNGKEYKCAVSNKALPAPIEKTISKAKGQPREPQVYTLPPSRDELTKNQVSLTCLVKGFYPSDIAVEWESNGQPENNYKTTPPVLDSDGSFFLYSKLTVDKSRWQQGNVFSCSVMHEALHNHYTQKSLSLSPGK

SEQ ID NO: 34 - protein, 214 aa, synthetic construct
  REGION 1..214: note = INX021 Variable Light with CDRs and affinity maturation mutated residues
DIVMTQSPSFLSASVGDRVTITCKASSNLGHAVAWYQQKPGKSPKLLIYSASNRYTGVPDRFSGSGSGTDFTLTISSLQPEDFADYFCQQYDDYPYTFGGGTKLEIKRTVAAPSVFIFPPSDEQLKSGTASVVCLLNNFYPREAKVQWKVDNALQSGNSQESVTEQDSKDSTYSLSSTLTLSKADYEKHKVYACEVTHQGLSSPVTKSFNRGEC